European Patent Application EP 4 796 126 A1, published August 26, 2026. Title: CLDN18_2抗体与化学治疗药物的组合及其应用. Applicant: 江苏奥赛康生物医药有限公司. The sequence listing filed with the application follows.

SEQUENCE LISTING (10 sequences)

SEQ ID NO: 1 - protein, 10 aa, synthetic construct
GYTFTSYVIN

SEQ ID NO: 2 - protein, 17 aa, synthetic construct
EIHPRGGNTYYSEKFRG

SEQ ID NO: 3 - protein, 9 aa, synthetic construct
LRRGNAMDY

SEQ ID NO: 4 - protein, 17 aa, synthetic construct
KSSQSLLNSGNQRNYLT

SEQ ID NO: 5 - protein, 7 aa, synthetic construct
WASTRES

SEQ ID NO: 6 - protein, 9 aa, synthetic construct
QNSYNYPYT

SEQ ID NO: 7 - protein, 118 aa, synthetic construct
QVQLVQSGAEVKKPGASVKVSCKASGYTFTSYVINWVRQATGQGLEWIGEIHPRGGNTYYSEKFRGRVTLTADTSISTAYMELSSLRSEDTAVYYCARLRRGNAMDYWDQGTTVTVSS

SEQ ID NO: 8 - protein, 113 aa, synthetic construct
DIVMTQSPSSLAVSLGEMATINCKSSQSLLNSGNQRNYLTWYQQKPGQPPKLLIYWASTRESGVPDRFSGSGSGTDFTLTISSLQAEDVAVYYCQNSYNYPYTFGQGTKLERK

SEQ ID NO: 9 - protein, 448 aa, synthetic construct
QVQLVQSGAEVKKPGASVKVSCKASGYTFTSYVINWVRQATGQGLEWIGEIHPRGGNTYYSEKFRGRVTLTADTSISTAYMELSSLRSEDTAVYYCARLRRGNAMDYWDQGTTVTVSSASTKGPSVFPLAPSSKSTSGGTAALGCLVKDYFPEPVTVSWNSGALTSGVHTFPAVLQSSGLYSLSSVVTVPSSSLGTQTYICNVNHKPSNTKVDKKVEPKSCDKTHTCPPCPAPELLGGPSVFLFPPKPKDTLMISRTPEVTCVVVDVSHEDPEVKFNWYVDGVEVHNAKTKPREEQYNSTYRVVSVLTVLHQDWLNGKEYKCKVSNKALPAPIEKTISKAKGQPREPQVYTLPPSRDELTKNQVSLTCLVKGFYPSDIAVEWESNGQPENNYKTTPPVLDSDGSFFLYSKLTVDKSRWQQGNVFSCSVMHEALHNHYTQKSLSLSPGK

SEQ ID NO: 10 - protein, 220 aa, synthetic construct
DIVMTQSPSSLAVSLGEMATINCKSSQSLLNSGNQRNYLTWYQQKPGQPPKLLIYWASTRESGVPDRFSGSGSGTDFTLTISSLQAEDVAVYYCQNSYNYPYTFGQGTKLERKRTVAAPSVFIFPPSDEQLKSGTASVVCLLNNFYPREAKVQWKVDNALQSGNSQESVTEQDSKDSTYSLSSTLTLSKADYEKHKVYACEVTHQGLSSPVTKSFNRGEC